European Patent Specification EP 3 555 124 B1, published May 1, 2024. Title: NYESO TCR. Applicant: Medigene Immunotherapies. The sequence listing filed with the application follows.

SEQUENCE LISTING (22 sequences)

SEQ ID NO: 1 - protein, 5 aa, Homo sapiens
LLMWI

SEQ ID NO: 2 - protein, 6 aa, Homo sapiens
SLLMWI

SEQ ID NO: 3 - protein, 9 aa, Homo sapiens
SLLMWITQC

SEQ ID NO: 4 - protein, 6 aa, Homo sapiens
DRGSQS

SEQ ID NO: 5 - protein, 6 aa, Homo sapiens
IYSNGD

SEQ ID NO: 6 - protein, 9 aa, Homo sapiens
CAADDKIIF

SEQ ID NO: 7 - protein, 5 aa, Homo sapiens
SGHDY

SEQ ID NO: 8 - protein, 6 aa, Homo sapiens
FNNNVP

SEQ ID NO: 9 - protein, 10 aa, Homo sapiens
CASSRGGSGY

SEQ ID NO: 10 - protein, 129 aa, Homo sapiens
MKSLRVLLVILWLQLSWVWSQQKEVEQNSGPLSVPEGAIASLNCTYSDRGSQSFFWYRQYSGKSPELIMFIYSNGDKEDGRFTAQLNKASQYVSLLIRDSQPSDSATYLCAADDKIIFGKGTRLHILPN

SEQ ID NO: 11 - protein, 132 aa, Homo sapiens
MGSWTLCCVSLCILVAKHTDAGVIQSPRHEVTEMGQEVTLRCKPISGHDYLFWYRQTMMRGLELLIYFNNNVPIDDSGMPEDRFSAKMPNASFSTLKIQPSEPRDSAVYFCASSRGGSGYTFGSGTRLTVVE

SEQ ID NO: 12 - protein, 269 aa, Homo sapiens
MKSLRVLLVILWLQLSWVWSQQKEVEQNSGPLSVPEGAIASLNCTYSDRGSQSFFWYRQYSGKSPELIMFIYSNGDKEDGRFTAQLNKASQYVSLLIRDSQPSDSATYLCAADDKIIFGKGTRLHILPNIQNPDPAVYQLRDSKSSDKSVCLFTDFDSQTNVSQSKDSDVYITDKTVLDMRSMDFKSNSAVAWSNKSDFACANAFNNSIIPEDTFFPSSDVPCDVKLVEKSFETDTNLNFQNLSVIGFRILLLKVAGFNLLMTLRLWSS

SEQ ID NO: 13 - protein, 308 aa, Homo sapiens
MGSWTLCCVSLCILVAKHTDAGVIQSPRHEVTEMGQEVTLRCKPISGHDYLFWYRQTMMRGLELLIYFNNNVPIDDSGMPEDRFSAKMPNASFSTLKIQPSEPRDSAVYFCASSRGGSGYTFGSGTRLTVVEDLNKVFPPEVAVFEPSKAEIAHTQKATLVCLATGFFPDHVELSWWVNGKEVHSGVSTDPQPLKEQPALNDSRYCLSSRLRVSATFWQNPRNHFRCQVQFYGLSENDEWTQDRAKPVTQIVSAEAWGRADCGITSASYHQGVLSATILYEILLGKATLYAVLVSALVLMAMVKRKDF

SEQ ID NO: 14 - protein, 180 aa, Homo sapiens
MQAEGRGTGGSTGDADGPGGPGIPDGPGGNAGGPGEAGATGGRGPRGAGAARASGPGGGAPRGPHGGAASGLNGCCRCGARGPESRLLEFYLAMPFATPMEAELARRSLAQDAPPLPVPGVLLKEFTVSGNILTIRLTAADHRQLQLSISSCLQQLSLLMWITQCFLPVFLAQPPSGQRR

SEQ ID NO: 15 - protein, 10 aa, Homo sapiens
FTVSGNILTI

SEQ ID NO: 16 - protein, 9 aa, Homo sapiens
RLLEFYLAM

SEQ ID NO: 17 - protein, 9 aa, Homo sapiens
ICLQWITQC

SEQ ID NO: 18 - protein, 9 aa, Homo sapiens
SLLFWILIC

SEQ ID NO: 19 - protein, 9 aa, Homo sapiens
SLLMWMLRL

SEQ ID NO: 20 - protein, 9 aa, Homo sapiens
NLLFWICGC

SEQ ID NO: 21 - protein, 9 aa, Homo sapiens
SLMYWITIQ

SEQ ID NO: 22 - protein, 9 aa, Homo sapiens
QLLGWITAH